European Patent Specification EP 3 585 814 B1, published December 10, 2025. Title: EGFR-BINDING AGENTS AND USES THEREOF. Applicant: University of Saskatchewan The Governing Council of the University of Toronto. The sequence listing filed with the application follows.

SEQUENCE LISTING (58 sequences)

SEQ ID NO: 1 - protein, 6 aa, Artificial Sequence
  Synthetic Construct
QSVSSA

SEQ ID NO: 2 - protein, 3 aa, Artificial Sequence
  Synthetic Construct
SAS

SEQ ID NO: 3 - protein, 9 aa, Artificial Sequence
  Synthetic Construct
QQWSYYPIT

SEQ ID NO: 4 - protein, 9 aa, Artificial Sequence
  Synthetic Construct
QQWSYYPFT

SEQ ID NO: 5 - protein, 8 aa, Artificial Sequence
  Synthetic Construct
QQSYWLIT

SEQ ID NO: 6 - protein, 9 aa, Artificial Sequence
  Synthetic Construct
GFNISSSSI

SEQ ID NO: 7 - protein, 9 aa, Artificial Sequence
  Synthetic Construct
GFNFSSSSI

SEQ ID NO: 8 - protein, 9 aa, Artificial Sequence
  Synthetic Construct
GFNLYSSSM

SEQ ID NO: 9 - protein, 10 aa, Artificial Sequence
  Synthetic Construct
YISSYYSSTY

SEQ ID NO: 10 - protein, 10 aa, Artificial Sequence
  Synthetic Construct
SIYPYSGYTY

SEQ ID NO: 11 - protein, 38 aa, Artificial Sequence
  Synthetic Construct
ARTYCPPLMLYNPTTYQMDVNPEGKYSFGATCGWAMDY

SEQ ID NO: 12 - protein, 38 aa, Artificial Sequence
  Synthetic Construct
ARTFCPPLMLYNPTTYQLEINPEAKYSFASTCGWAMDY

SEQ ID NO: 13 - protein, 38 aa, Artificial Sequence
  Synthetic Construct
ARTFCPPIMLFNATSFELDIDAEAKFSFASTCGWAMDY

SEQ ID NO: 14 - protein, 38 aa, Artificial Sequence
  Synthetic Construct
ARTFCPPLMLFNPTTFQLEINAEAKYSFASTCGWAMDY

SEQ ID NO: 15 - protein, 38 aa, Artificial Sequence
  Synthetic Construct
ARTYCPPLMRYNPTTYQMDVNPEAQYSFGATCGWAMDY

SEQ ID NO: 16 - protein, 15 aa, Artificial Sequence
  Synthetic Construct
ARYPFGVSAYYAMDY

SEQ ID NO: 17 - protein, 6 aa, Artificial Sequence
  Synthetic Construct
SSYSLI

SEQ ID NO: 18 - protein, 6 aa, Artificial Sequence
  Synthetic Construct
FSSSSI

SEQ ID NO: 19 - protein, 10 aa, Artificial Sequence
  Synthetic Construct
SISSSYGYTY

SEQ ID NO: 20 - protein, 15 aa, Artificial Sequence
  Synthetic Construct
TVRGSKKPYFSGWAM

SEQ ID NO: 21 - protein, 6 aa, Artificial Sequence
  Synthetic Construct
WSYYPI

SEQ ID NO: 22 - protein, 6 aa, Artificial Sequence
  Synthetic Construct
ISSSSI

SEQ ID NO: 23 - protein, 10 aa, Artificial Sequence
  Synthetic Construct
YISSYYSSTY

SEQ ID NO: 24 - protein, 34 aa, Artificial Sequence
  Synthetic Construct
TYCPPLMLYNPTTYQMDVNPEGKYSFGATCGWAM

SEQ ID NO: 25 - protein, 6 aa, Artificial Sequence
  Synthetic Construct
WSYYPI

SEQ ID NO: 26 - protein, 6 aa, Artificial Sequence
  Synthetic Construct
ISSSSI

SEQ ID NO: 27 - protein, 10 aa, Artificial Sequence
  Synthetic Construct
YISSYYSSTY

SEQ ID NO: 28 - protein, 34 aa, Artificial Sequence
  Synthetic Construct
TYCPPLMRYNPTTYQMDVNPEAQYSFGATCGWAM

SEQ ID NO: 29 - protein, 5 aa, Artificial Sequence
  Synthetic Construct
SYWLI

SEQ ID NO: 30 - protein, 6 aa, Artificial Sequence
  Synthetic Construct
LYSSSM

SEQ ID NO: 31 - protein, 10 aa, Artificial Sequence
  Synthetic Construct
SIYPYSGYTY

SEQ ID NO: 32 - protein, 11 aa, Artificial Sequence
  Synthetic Construct
YPFGVSAYYAM

SEQ ID NO: 33 - DNA, 762 bp, Artificial Sequence
  Synthetic Construct
gaggttcagctggtggagtctggcggtggcctggtgcagccagggggctcactccgtttgtcctgtgcagcttctggcttcaacatctcttcttcttctatccactgggtgcgtcaggccccgggtaagggcctggaatgggttgcatatatttcttcttattatagctctacttattatgccgatagcgtcaagggccgtttcactataagcgcagacacatccaaaaacacagcctacctacaaatgaacagcctgagagctgaggacactgccgtctattattgtgctcgcacttactgtccccccctgatgctgtacaaccccactacttaccaaatggacgtcaaccccgaaggtaaatactcttttggtgctacttgtggctgggctatggactactggggtcaaggaaccctggtcaccgtctcctcggcctccaccaagggcccatcggtcttccccctggcaccctcctccaagagcacctctgggggcacagcggccctgggctgcctggtcaaggactacttccccgaaccggtgacggtgtcgtggaactcaggcgccctgaccagcggcgtgcacaccttcccggctgtcctacagtcctcaggactctactccctcagcagcgtggtgaccgtgccctccagcagcttgggcacccagacctacatctgcaacgtgaatcacaagcccagcaacaccaaggtcgacaagaaagttgagcccaaatcttgtgacaaaactcacacataa

SEQ ID NO: 34 - protein, 253 aa, Artificial Sequence
  Synthetic Construct
EVQLVESGGGLVQPGGSLRLSCAASGFNISSSSIHWVRQAPGKGLEWVAYISSYYSSTYYADSVKGRFTISADTSKNTAYLQMNSLRAEDTAVYYCARTYCPPLMLYNPTTYQMDVNPEGKYSFGATCGWAMDYWGQGTLVTVSSASTKGPSVFPLAPSSKSTSGGTAALGCLVKDYFPEPVTVSWNSGALTSGVHTFPAVLQSSGLYSLSSVVTVPSSSLGTQTYICNVNHKPSNTKVDKKVEPKSCDKTHT

SEQ ID NO: 35 - DNA, 678 bp, Artificial Sequence
  Synthetic Construct
gatatccagatgacccagtccccgagctccctgtccgcctctgtgggcgatagggtcaccatcacctgccgtgccagtcagtccgtgtccagcgctgtagcctggtatcaacagaaaccaggaaaagctccgaagcttctgatttactcggcatccagcctctactctggagtcccttctcgcttctctggtagccgttccgggacggatttcactctgaccatcagcagtctgcagccggaagacttcgcaacttattactgtcagcaatggtcttactacccgatcacgttcggacagggtaccaaggtggagatcaaacgaactgtggctgcaccatctgtcttcatcttcccgccatctgattcacagcttaagtctggaactgcctctgttgtgtgcctgctgaataacttctatcccagagaggccaaagtacagtggaaggtggataacgccctccaatcgggtaactcccaggagagtgtcacagagcaggacagcaaggacagcacctacagcctcagcagcaccctgacgctgagcaaagcagactacgaaaaacataaagtctacgcctgcgaagtcacccatcagggcctgagctcgcccgtcacaaagagcttcaacaggggagagtgtggtggttctgattacaaagatgacgatgacaaataa

SEQ ID NO: 36 - protein, 225 aa, Artificial Sequence
  Synthetic Construct
DIQMTQSPSSLSASVGDRVTITCRASQSVSSAVAWYQQKPGKAPKLLIYSASSLYSGVPSRFSGSRSGTDFTLTISSLQPEDFATYYCQQWSYYPITFGQGTKVEIKRTVAAPSVFIFPPSDSQLKSGTASVVCLLNNFYPREAKVQWKVDNALQSGNSQESVTEQDSKDSTYSLSSTLTLSKADYEKHKVYACEVTHQGLSSPVTKSFNRGECGGSDYKDDDDK

SEQ ID NO: 37 - DNA, 762 bp, Artificial Sequence
  Synthetic Construct
gaggttcagctggtggagtctggcggtggcctggtgcagccagggggctcactccgtttgtcctgtgcagcttctggcttcaacatctcttcttcttctatccactgggtgcgtcaggccccgggtaagggcctggaatgggttgcatatatttcttcttattatagctctacttattatgccgatagcgtcaagggccgtttcactataagcgcagacacatccaaaaacacagcctacctacaaatgaacagcctgagagctgaggacactgccgtctattattgtgctcgcactttctgcccaccactcatgctctacaacccaaccacctaccaactggaaattaacccagaagctaagtactccttcgcttctacctgcggttgggctatggactactggggtcaaggaaccctggtcaccgtctcctcggcctccaccaagggcccatcggtcttccccctggcaccctcctccaagagcacctctgggggcacagcggccctgggctgcctggtcaaggactacttcccggaaccggtgacggtgtcgtggaactcaggcgccctgaccagcggcgtgcacaccttcccggctgtcctacagtcctcaggactctactccctcagcagcgtggtgaccgtgccctccagcagcttgggcacccagacctacatctgcaacgtgaatcacaagcccagcaacaccaaggtcgacaagaaagttgagcccaaatcttgtgacaaaactcacacataa

SEQ ID NO: 38 - protein, 253 aa, Artificial Sequence
  Synthetic Construct
EVQLVESGGGLVQPGGSLRLSCAASGFNISSSSIHWVRQAPGKGLEWVAYISSYYSSTYYADSVKGRFTISADTSKNTAYLQMNSLRAEDTAVYYCARTFCPPLMLYNPTTYQLEINPEAKYSFASTCGWAMDYWGQGTLVTVSSASTKGPSVFPLAPSSKSTSGGTAALGCLVKDYFPEPVTVSWNSGALTSGVHTFPAVLQSSGLYSLSSVVTVPSSSLGTQTYICNVNHKPSNTKVDKKVEPKSCDKTHT

SEQ ID NO: 39 - DNA, 678 bp, Artificial Sequence; identical to SEQ ID NO: 35
  Synthetic Construct

SEQ ID NO: 40 - protein, 225 aa, Artificial Sequence; identical to SEQ ID NO: 36
  Synthetic Construct

SEQ ID NO: 41 - DNA, 762 bp, Artificial Sequence
  Synthetic Construct
gaggttcagctggtggagtctggcggtggcctggtgcagccagggggctcactccgtttgtcctgtgcagcttctggcttcaacatctcttcttcttctatccactgggtgcgtcaggccccgggtaagggcctggaatgggttgcatatatttcttcttattatagctctacttattatgccgatagcgtcaagggccgtttcactataagcgcagacacatccaaaaacacagcctacctacaaatgaacagcctgagagctgaggacactgccgtctattattgtgctcgcactttctgcccaccaatcatgctcttcaacgcaaccagcttcgaactggacattgacgcagaagctaagttctccttcgcttctacctgcggttgggctatggactactggggtcaaggaaccctggtcaccgtctcctcggcctccaccaagggcccatcggtcttccccctggcaccctcctccaagagcacctctgggggcacagcggccctgggctgcctggtcaaggactacttcccggaaccggtgacggtgtcgtggaactcaggcgccctgaccagcggcgtgcacaccttcccggctgtcctacagtcctcaggactctactccctcagcagcgtggtgaccgtgccctccagcagcttgggcacccagacctacatctgcaacgtgaatcacaagcccagcaacaccaaggtcgacaagaaagttgagcccaaatcttgtgacaaaactcacacataa

SEQ ID NO: 42 - protein, 253 aa, Artificial Sequence
  Synthetic Construct
EVQLVESGGGLVQPGGSLRLSCAASGFNISSSSIHWVRQAPGKGLEWVAYISSYYSSTYYADSVKGRFTISADTSKNTAYLQMNSLRAEDTAVYYCARTFCPPIMLFNATSFELDIDAEAKFSFASTCGWAMDYWGQGTLVTVSSASTKGPSVFPLAPSSKSTSGGTAALGCLVKDYFPEPVTVSWNSGALTSGVHTFPAVLQSSGLYSLSSVVTVPSSSLGTQTYICNVNHKPSNTKVDKKVEPKSCDKTHT

SEQ ID NO: 43 - DNA, 678 bp, Artificial Sequence; identical to SEQ ID NO: 35
  Synthetic Construct

SEQ ID NO: 44 - protein, 225 aa, Artificial Sequence; identical to SEQ ID NO: 36
  Synthetic Construct

SEQ ID NO: 45 - DNA, 762 bp, Artificial Sequence
  Synthetic Construct
gaggttcagctggtggagtctggcggtggcctggtgcagccagggggctcactccgtttgtcctgtgcagcttctggcttcaacatctcttcttcttctatccactgggtgcgtcaggccccgggtaagggcctggaatgggttgcatatatttcttcttattatagctctacttattatgccgatagcgtcaagggccgtttcactataagcgcagacacatccaaaaacacagcctacctacaaatgaacagcctgagagctgaggacactgccgtctattattgtgctcgcactttctgcccaccactcatgctcttcaacccaaccaccttccaactggaaattaacgcagaagctaagtactccttcgcttctacctgcggttgggctatggactactggggtcaaggaaccctggtcaccgtctcctcggcctccaccaagggcccatcggtcttccccctggcaccctcctccaagagcacctctgggggcacagcggccctgggctgcctggtcaaggactacttccccgaaccggtgacggtgtcgtggaactcaggcgccctgaccagcggcgtgcacaccttcccggctgtcctacagtcctcaggactctactccctcagcagcgtggtgaccgtgccctccagcagcttgggcacccagacctacatctgcaacgtgaatcacaagcccagcaacaccaaggtcgacaagaaagttgagcccaaatcttgtgacaaaactcacacataa

SEQ ID NO: 46 - protein, 253 aa, Artificial Sequence
  Synthetic Construct
EVQLVESGGGLVQPGGSLRLSCAASGFNISSSSIHWVRQAPGKGLEWVAYISSYYSSTYYADSVKGRFTISADTSKNTAYLQMNSLRAEDTAVYYCARTFCPPLMLFNPTTFQLEINAEAKYSFASTCGWAMDYWGQGTLVTVSSASTKGPSVFPLAPSSKSTSGGTAALGCLVKDYFPEPVTVSWNSGALTSGVHTFPAVLQSSGLYSLSSVVTVPSSSLGTQTYICNVNHKPSNTKVDKKVEPKSCDKTHT

SEQ ID NO: 47 - DNA, 678 bp, Artificial Sequence
  Synthetic Construct
gatatccagatgacccagtccccgagctccctgtccgcctctgtgggcgatagggtcaccatcacctgccgtgccagtcagtccgtgtccagcgctgtagcctggtatcaacagaaaccaggaaaagctccgaagcttctgatttactcggcatccagcctctactctggagtcccttctcgcttctctggtagccgttccgggacggatttcactctgaccatcagcagtctgcagccggaagacttcgcaacttattactgtcagcaatggtcttactacccgatcacgttcggacagggtaccaaggtggagatcaaacgaactgtggctgcaccatctgtcttcatcttcccgccatctgattcacagttgaaatctggaactgcctctgttgtgtgcctgctgaataacttctatcccagagaggccaaagtacagtggaaggtggataacgccctccaatcgggtaactcccaggagagtgtcacagagcaggacagcaaggacagcacctacagcctcagcagcaccctgacgctgagcaaagcagactacgaaaaacataaagtctacgcctgcgaagtcacccatcagggcctgagctcgcccgtcacaaagagcttcaacaggggagagtgtggtggttctgattacaaagatgacgatgacaaataa

SEQ ID NO: 48 - protein, 225 aa, Artificial Sequence; identical to SEQ ID NO: 36
  Synthetic Construct

SEQ ID NO: 49 - DNA, 762 bp, Artificial Sequence
  Synthetic Construct
gaggttcagctggtggagtctggcggtggcctggtgcagccagggggctcactccgtttgtcctgtgcagcttctggcttcaacatctcttcttcttctatccactgggtgcgtcaggccccgggtaagggcctggaatgggttgcatatatttcttcttattatagctctacttattatgccgatagcgtcaagggccgtttcactataagcgcagacacatccaaaaacacagcctacctacaaatgaacagcctgagagctgaggacactgccgtctattattgtgctcgcacttactgtccccccctgatgcggtacaaccccactacttaccaaatggacgtcaaccccgaggctcaatactcttttggggctacttgtggctgggctatggactactggggtcaaggaaccctggtcaccgtctcctcggcctccaccaagggcccatcggtcttccccctggcaccctcctccaagagcacctctgggggcacagcggccctgggctgcctggtcaaggactacttcccggaaccggtgacggtgtcgtggaactcaggcgccctgaccagcggcgtgcacaccttcccggctgtcctacagtcctcaggactctactccctcagcagcgtggtgaccgtgccctccagcagcttgggcacccagacctacatctgcaacgtgaatcacaagcccagcaacaccaaggtcgacaagaaagttgagcccaaatcttgtgacaaaactcacacataa

SEQ ID NO: 50 - protein, 253 aa, Artificial Sequence
  Synthetic Construct
EVQLVESGGGLVQPGGSLRLSCAASGFNISSSSIHWVRQAPGKGLEWVAYISSYYSSTYYADSVKGRFTISADTSKNTAYLQMNSLRAEDTAVYYCARTYCPPLMRYNPTTYQMDVNPEAQYSFGATCGWAMDYWGQGTLVTVSSASTKGPSVFPLAPSSKSTSGGTAALGCLVKDYFPEPVTVSWNSGALTSGVHTFPAVLQSSGLYSLSSVVTVPSSSLGTQTYICNVNHKPSNTKVDKKVEPKSCDKTHT

SEQ ID NO: 51 - DNA, 678 bp, Artificial Sequence; identical to SEQ ID NO: 47
  Synthetic Construct

SEQ ID NO: 52 - protein, 225 aa, Artificial Sequence; identical to SEQ ID NO: 36
  Synthetic Construct

SEQ ID NO: 53 - DNA, 693 bp, Artificial Sequence
  Synthetic Construct
gaggttcagctggtggagtctggcggtggcctggtgcagccagggggctcactccgtttgtcctgtgcagcttctggcttcaacctctattcttcttctatgcactgggtgcgtcaggccccgggtaagggcctggaatgggttgcatctatttatccttattctggctatacttattatgccgatagcgtcaagggccgtttcactataagcgcagacacatccaaaaacacagcctacctacaaatgaacagcttaagagctgaggacactgccgtctattattgtgctcgctacccgttcggtgtttctgcttactacgctatggactactggggtcaaggaaccctggtcaccgtctcctcggcctccaccaagggtccatcggtcttccccctggcaccctcctccaagagcacctctgggggcacagcggccctgggctgcctggtcaaggactacttccccgaaccggtgacggtgtcgtggaactcaggcgccctgaccagcggcgtgcacaccttcccggctgtcctacagtcctcaggactctactccctcagcagcgtggtgaccgtgccctccagcagcttgggcacccagacctacatctgcaacgtgaatcacaagcccagcaacaccaaggtcgacaagaaagttgagcccaaatcttgtgacaaaactcacacataa

SEQ ID NO: 54 - protein, 230 aa, Artificial Sequence
  Synthetic Construct
EVQLVESGGGLVQPGGSLRLSCAASGFNLYSSSMHWVRQAPGKGLEWVASIYPYSGYTYYADSVKGRFTISADTSKNTAYLQMNSLRAEDTAVYYCARYPFGVSAYYAMDYWGQGTLVTVSSASTKGPSVFPLAPSSKSTSGGTAALGCLVKDYFPEPVTVSWNSGALTSGVHTFPAVLQSSGLYSLSSVVTVPSSSLGTQTYICNVNHKPSNTKVDKKVEPKSCDKTHT

SEQ ID NO: 55 - DNA, 675 bp, Artificial Sequence
  Synthetic Construct
gatatccagatgacccagtccccgagctccctgtccgcctctgtgggcgatagggtcaccatcacctgccgtgccagtcagtccgtgtccagcgctgtagcctggtatcaacagaaaccaggaaaagctccgaagcttctgatttactcggcatccagcctctactctggagtcccttctcgcttctctggtagccgttccgggacggatttcactctgaccatcagcagtctgcagccggaagacttcgcaacttattactgtcagcaatcttactggctgatcacgttcggacagggtaccaaggtggagatcaaacgaactgtggctgcaccatctgtcttcatcttcccgccatctgattcacagttgaaatctggaactgcctctgttgtgtgcctgctgaataacttctatcccagagaggccaaagtacagtggaaggtggataacgccctccaatcgggtaactcccaggagagtgtcacagagcaggacagcaaggacagcacctacagcctcagcagcaccctgacgctgagcaaagcagactacgaaaaacataaagtctacgcctgcgaagtcacccatcagggcctgagctcgcccgtcacaaagagcttcaacaggggagagtgtggtggttctgattacaaagatgacgatgacaaataa

SEQ ID NO: 56 - protein, 224 aa, Artificial Sequence
  Synthetic Construct
DIQMTQSPSSLSASVGDRVTITCRASQSVSSAVAWYQQKPGKAPKLLIYSASSLYSGVPSRFSGSRSGTDFTLTISSLQPEDFATYYCQQSYWLITFGQGTKVEIKRTVAAPSVFIFPPSDSQLKSGTASVVCLLNNFYPREAKVQWKVDNALQSGNSQESVTEQDSKDSTYSLSSTLTLSKADYEKHKVYACEVTHQGLSSPVTKSFNRGECGGSDYKDDDDK

SEQ ID NO: 57 - protein, 28 aa, Artificial Sequence
  Synthetic Construct
CPPLMLYNPTTYQMDVNPEGKYSFGATC

SEQ ID NO: 58 - protein, 15 aa, Artificial Sequence
  Synthetic Construct
TVRGSKKPYFSGWAM